European Patent Specification EP 3 577 462 B1, published April 17, 2024. Title: C PEPTIDE’S INTERACTION WITH ELASTIN RECEPTOR, A BLUEPRINT FOR UNDERSTANDING VASCULAR DISEASE. Applicant: Wensvoort Gert RESILIUN B.V. The sequence listing filed with the application follows.

SEQUENCE LISTING (230 sequences)

SEQ ID NO: 1 - protein, 31 aa, Homo sapiens
EAEDLQVGQVELGGGPGAGSLQPLALEGSLQ

SEQ ID NO: 2 - protein, 12 aa, Homo sapiens
EAEDLQVGQVEL

SEQ ID NO: 3 - protein, 13 aa, Homo sapiens
GGGPGAGSLQPLA

SEQ ID NO: 4 - protein, 6 aa, Homo sapiens
LEGSLQ

SEQ ID NO: 5 - protein, 4 aa, Homo sapiens
EAED

SEQ ID NO: 6 - protein, 5 aa, Homo sapiens
EGSLQ

SEQ ID NO: 7 - protein, 5 aa, Rattus norvegicus
EVARQ

SEQ ID NO: 8 - protein, 7 aa, Homo sapiens
GGGPGAG

SEQ ID NO: 9 - protein, 9 aa, Homo sapiens
ELGGGPGAG

SEQ ID NO: 10 - protein, 28 aa, Homo sapiens
DLQVGQVELGGGPGAGSLQPLALEGSLQ

SEQ ID NO: 11 - protein, 27 aa, Homo sapiens
LQVGQVELGGGPGAGSLQPLALEGSLQ

SEQ ID NO: 12 - protein, 25 aa, Homo sapiens
VGQVELGGGPGAGSLQPLALEGSLQ

SEQ ID NO: 13 - protein, 24 aa, Homo sapiens
GQVELGGGPGAGSLQPLALEGSLQ

SEQ ID NO: 14 - protein, 20 aa, Homo sapiens
LGGGPGAGSLQPLALEGSLQ

SEQ ID NO: 15 - protein, 20 aa, Homo sapiens
VGQVELGGGPGAGSLQPLAL

SEQ ID NO: 16 - protein, 19 aa, Homo sapiens
EVGQVELGGGPGAGSLQPL

SEQ ID NO: 17 - protein, 26 aa, Homo sapiens
EAEDLQVGQVELGGGPGAGSLQPLAL

SEQ ID NO: 18 - protein, 24 aa, Homo sapiens
EAEDLQVGQVELGGGPGAGSLQPL

SEQ ID NO: 19 - protein, 22 aa, Homo sapiens
LQVGQVELGGGPGAGSLQPLAL

SEQ ID NO: 20 - protein, 21 aa, Homo sapiens
DLQVGQVELGGGPGAGSLQPL

SEQ ID NO: 21 - protein, 20 aa, Homo sapiens
LQVGQVELGGGPGAGSLQPL

SEQ ID NO: 22 - protein, 13 aa, Homo sapiens
LGGGPGAGSLQPL

SEQ ID NO: 23 - protein, 15 aa, Homo sapiens
VGQVELGGGPGAGSL

SEQ ID NO: 24 - protein, 10 aa, Homo sapiens
GGGPGAGSLQ

SEQ ID NO: 25 - protein, 19 aa, Homo sapiens
FRAAPLQGMLPGLLAPLRT

SEQ ID NO: 26 - protein, 15 aa, Homo sapiens
AAPLQGMLPGLLAPL

SEQ ID NO: 27 - protein, 12 aa, Homo sapiens
LQGMLPGLLAPL

SEQ ID NO: 28 - protein, 10 aa, Homo sapiens
LQGMLPGLLA

SEQ ID NO: 29 - protein, 7 aa, Homo sapiens
LQGMLPG

SEQ ID NO: 30 - protein, 8 aa, Homo sapiens
GMLPGLLA

SEQ ID NO: 31 - protein, 4 aa, Homo sapiens
QDEA

SEQ ID NO: 32 - protein, 8 aa, Homo sapiens
LGGGPGAG

SEQ ID NO: 33 - protein, 8 aa, Bos taurus
LAGGPGAG

SEQ ID NO: 34 - protein, 6 aa, Homo sapiens
LGGGPG

SEQ ID NO: 35 - protein, 6 aa, Bos taurus
LAGGPG

SEQ ID NO: 36 - protein, 5 aa, Homo sapiens
LGGGP

SEQ ID NO: 37 - protein, 5 aa, Bos taurus
LAGGP

SEQ ID NO: 38 - protein, 4 aa, Homo sapiens
GGGP

SEQ ID NO: 39 - protein, 4 aa, Artificial Sequence
  Retro sequence peptide
GAGP

SEQ ID NO: 40 - protein, 5 aa, Homo sapiens
GGGPG

SEQ ID NO: 41 - protein, 6 aa, Homo sapiens
VGVAPG

SEQ ID NO: 42 - protein, 10 aa, Homo sapiens
ELGGGPGAGS

SEQ ID NO: 43 - protein, 6 aa, Artificial Sequence
  Immunomodulatory peptide
QGQLPG

SEQ ID NO: 44 - protein, 6 aa, Homo sapiens
  selected from human Galectin-3
PGAYPG

SEQ ID NO: 45 - protein, 6 aa, Homo sapiens
  selected from loop 2 of human beta-hCG
QGVLPA

SEQ ID NO: 46 - protein, 5 aa, Bos taurus
GAGPG

SEQ ID NO: 47 - protein, 7 aa, Homo sapiens
LGGGPGA

SEQ ID NO: 48 - protein, 6 aa, Homo sapiens
GGPGAG

SEQ ID NO: 49 - protein, 6 aa, Homo sapiens
GGGPGA

SEQ ID NO: 50 - protein, 5 aa, Homo sapiens
GGGPE

SEQ ID NO: 51 - protein, 5 aa, Homo sapiens
GAIPG

SEQ ID NO: 52 - protein, 5 aa, Homo sapiens
GGVPG

SEQ ID NO: 53 - protein, 5 aa, Homo sapiens
GVAPG

SEQ ID NO: 54 - protein, 14 aa, Homo sapiens
YTTGKLPYGYGPGG

SEQ ID NO: 55 - protein, 12 aa, Homo sapiens
YGARPGVGVGIP

SEQ ID NO: 56 - protein, 9 aa, Homo sapiens
PGFGAVPGA

SEQ ID NO: 57 - protein, 5 aa, Homo sapiens
GVYPG

SEQ ID NO: 58 - protein, 5 aa, Homo sapiens
GFGPG

SEQ ID NO: 59 - protein, 5 aa, Homo sapiens
GVLPG

SEQ ID NO: 60 - protein, 6 aa, Homo sapiens
PGAIPG

SEQ ID NO: 61 - protein, 6 aa, Homo sapiens
PGAVGP

SEQ ID NO: 62 - protein, 6 aa, Homo sapiens
VGAMPG

SEQ ID NO: 63 - protein, 6 aa, Homo sapiens
VGSLPG

SEQ ID NO: 64 - protein, 6 aa, Homo sapiens
VGMAPG

SEQ ID NO: 65 - protein, 5 aa, Homo sapiens
VPGVG

SEQ ID NO: 66 - protein, 5 aa, Homo sapiens
IPGVG

SEQ ID NO: 67 - protein, 5 aa, Homo sapiens
VGVPG

SEQ ID NO: 68 - protein, 6 aa, Homo sapiens
AGAIPG

SEQ ID NO: 69 - protein, 4 aa, Homo sapiens
VPGV

SEQ ID NO: 70 - protein, 6 aa, Homo sapiens
LGITPG

SEQ ID NO: 71 - protein, 4 aa, Homo sapiens
GDNP

SEQ ID NO: 72 - protein, 4 aa, Homo sapiens
GAIP

SEQ ID NO: 73 - protein, 4 aa, Homo sapiens
GKVP

SEQ ID NO: 74 - protein, 4 aa, Homo sapiens
GVQY

SEQ ID NO: 75 - protein, 4 aa, Homo sapiens
GVLP

SEQ ID NO: 76 - protein, 4 aa, Homo sapiens
GVGP

SEQ ID NO: 77 - protein, 4 aa, Homo sapiens
GFGP

SEQ ID NO: 78 - protein, 4 aa, Homo sapiens
GGIP

SEQ ID NO: 79 - protein, 4 aa, Homo sapiens
GVAP

SEQ ID NO: 80 - protein, 4 aa, Homo sapiens
GIGP

SEQ ID NO: 81 - protein, 5 aa, Homo sapiens
GGIPP

SEQ ID NO: 82 - protein, 4 aa, Homo sapiens
GQFP

SEQ ID NO: 83 - protein, 4 aa, Homo sapiens
GLSP

SEQ ID NO: 84 - protein, 4 aa, Homo sapiens
GPQP

SEQ ID NO: 85 - protein, 5 aa, Homo sapiens
GGPQP

SEQ ID NO: 86 - protein, 5 aa, Homo sapiens
GPQPG

SEQ ID NO: 87 - protein, 6 aa, Homo sapiens
GGPQPG

SEQ ID NO: 88 - protein, 4 aa, Homo sapiens
GIPP

SEQ ID NO: 89 - protein, 5 aa, Homo sapiens
GIPPA

SEQ ID NO: 90 - protein, 6 aa, Homo sapiens
GGIPPA

SEQ ID NO: 91 - protein, 58 aa, Homo sapiens
GGYPGASYPGAYPGQAPPGAYPGQAPPGAYPGAPGAYPGAPAPGVYPGPPSGPGAYPS

SEQ ID NO: 92 - protein, 9 aa, Homo sapiens
GGYPGASYP

SEQ ID NO: 93 - protein, 9 aa, Homo sapiens
GAYPGQAPP

SEQ ID NO: 94 - protein, 7 aa, Homo sapiens
GAYPGQA

SEQ ID NO: 95 - protein, 7 aa, Homo sapiens
GAYPGAP

SEQ ID NO: 96 - protein, 5 aa, Homo sapiens
GAYPG

SEQ ID NO: 97 - protein, 9 aa, Homo sapiens
APAPGVYPG

SEQ ID NO: 98 - protein, 5 aa, Homo sapiens
GAYPS

SEQ ID NO: 99 - protein, 40 aa, Homo sapiens
QTLPGSCGQVVGSPSAQDEASPLSEWRASYNSAGSNITDA

SEQ ID NO: 100 - protein, 32 aa, Homo sapiens
LPGSCGQVVGSPSAQDEASPLSEWRASYNSAG

SEQ ID NO: 101 - protein, 21 aa, Homo sapiens
VVGSPSAQDEASPLSEWRASY

SEQ ID NO: 102 - protein, 15 aa, Homo sapiens
VVGSPSAQDEASPLS

SEQ ID NO: 103 - protein, 10 aa, Homo sapiens
PSAQDEASPL

SEQ ID NO: 104 - protein, 10 aa, Homo sapiens
SPSAQDEASP

SEQ ID NO: 105 - protein, 6 aa, Homo sapiens
AQDEAS

SEQ ID NO: 106 - protein, 4 aa, Homo sapiens
PSAQ

SEQ ID NO: 107 - protein, 4 aa, Homo sapiens
SAQD

SEQ ID NO: 108 - protein, 4 aa, Homo sapiens
DEAS

SEQ ID NO: 109 - protein, 4 aa, Homo sapiens
SPSA

SEQ ID NO: 110 - protein, 15 aa, Artificial Sequence
  antagonist peptide
VVGGTEAQRNSWPLQ

SEQ ID NO: 111 - protein, 15 aa, Artificial Sequence
  antagonist peptide
VVGGTEAQRNSWPSQ

SEQ ID NO: 112 - protein, 9 aa, Artificial Sequence
  antagonist peptide
TEAQRNSWP

SEQ ID NO: 113 - protein, 4 aa, Artificial Sequence
  antagonist peptide
AQRN

SEQ ID NO: 114 - protein, 15 aa, Artificial Sequence
  antagonist peptide
IVGGRRARPHAWPFM

SEQ ID NO: 115 - protein, 15 aa, Artificial Sequence
  antagonist peptide
VVGGEDAKPGQFPWQ

SEQ ID NO: 116 - protein, 15 aa, Artificial Sequence
  antagonist peptide
VVGGRVAQPNSWPWQ

SEQ ID NO: 117 - protein, 8 aa, Artificial Sequence
  antagonist peptide
RVAQPNSW

SEQ ID NO: 118 - protein, 15 aa, Artificial Sequence
  antagonist peptide
VVGGAEARRNSWPSQ

SEQ ID NO: 119 - protein, 8 aa, Artificial Sequence
  antagonist peptide
AEARRNSW

SEQ ID NO: 120 - protein, 15 aa, Artificial Sequence
  antagonist peptide
VVGGQEATPNTWPWQ

SEQ ID NO: 121 - protein, 8 aa, Artificial Sequence
  antagonist peptide
QEATPNTW

SEQ ID NO: 122 - protein, 15 aa, Artificial Sequence
  antagonist peptide
VVGGEEARPNSWPWQ

SEQ ID NO: 123 - protein, 8 aa, Artificial Sequence
  antagonist peptide
EEARPNSW

SEQ ID NO: 124 - protein, 15 aa, Artificial Sequence
  antagonist
VVGGTEAGRNSWPSQ

SEQ ID NO: 125 - protein, 9 aa, Artificial Sequence
  antagonist
TEAGRNSWP

SEQ ID NO: 126 - protein, 15 aa, Artificial Sequence
  antagonist peptide
EDYRPSQQDECSPRE

SEQ ID NO: 127 - protein, 9 aa, Artificial Sequence
  antagonist peptide
PSQQDECSP

SEQ ID NO: 128 - protein, 5 aa, Artificial Sequence
  antagonist peptide
QQDEC

SEQ ID NO: 129 - protein, 8 aa, Homo sapiens
LALEGSLQ

SEQ ID NO: 130 - protein, 4 aa, Homo sapiens
AGGP

SEQ ID NO: 131 - protein, 14 aa, Homo sapiens
VVGSPSAQDEASPL

SEQ ID NO: 132 - skipped

SEQ ID NO: 133 - protein, 7 aa, Homo sapiens
GGGPGAG

SEQ ID NO: 134 - protein, 6 aa, Rattus norvegicus
LGGGPE

SEQ ID NO: 135 - protein, 6 aa, Sus scrofa
LGGGLG

SEQ ID NO: 136 - protein, 31 aa, Artificial Sequence
  retro C-Peptide
QLSGELALPQLSGAGPGGGLEVQGVQLDEAE

SEQ ID NO: 137 - protein, 6 aa, Homo sapiens
LGTIPG

SEQ ID NO: 138 - protein, 6 aa, Artificial Sequence
  scrambled peptide
GVAPGV

SEQ ID NO: 139 - protein, 6 aa, Artificial Sequence
  scrambled peptide
VAPGVG

SEQ ID NO: 140 - protein, 6 aa, Artificial Sequence
  scrambled peptide
APGVGV

SEQ ID NO: 141 - protein, 6 aa, Artificial Sequence
  scrambled peptide
PGVGVA

SEQ ID NO: 142 - protein, 6 aa, Artificial Sequence
  scrambled peptide
GVGVAP

SEQ ID NO: 143 - protein, 10 aa, Homo sapiens
VPGVGISPEA

SEQ ID NO: 144 - protein, 10 aa, Homo sapiens
GVAPGIGPGG

SEQ ID NO: 145 - protein, 14 aa, Homo sapiens
VELGGGPGAGSLQP

SEQ ID NO: 146 - protein, 12 aa, Homo sapiens
LGGGPGAGSLQP

SEQ ID NO: 147 - protein, 9 aa, Homo sapiens
LGGGPGAGS

SEQ ID NO: 148 - protein, 55 aa, Homo sapiens
AGAGGYPGASYPGAYPGQAPPGAYPGQAPPGAYPGAPGAYPGAPAPGVYPGPPSG

SEQ ID NO: 149 - protein, 6 aa, Homo sapiens
EGFEPG

SEQ ID NO: 150 - protein, 31 aa, Homo sapiens
EAEDLQVGQVEMGGGPGAGSLQPLALEGSLQ

SEQ ID NO: 151 - protein, 31 aa, Homo sapiens
EAEDLQVGQVELGGGPGAGSLQPLALERSLQ

SEQ ID NO: 152 - protein, 31 aa, Hylobatidae
EAEDPQVGQVELGGGPGAGSLQPLALEGSLQ

SEQ ID NO: 153 - protein, 31 aa, Mus musculus
EVEDPQVAQLELGGGPGAGDLQTLALEVAQQ

SEQ ID NO: 154 - protein, 31 aa, Rattus norvegicus
EVEDPQVAQLELGGGPGAGDLQTLALEVARQ

SEQ ID NO: 155 - protein, 31 aa, Rattus norvegicus
EVEDPQVPQLELGGGPEAGDLQTLALEVARQ

SEQ ID NO: 156 - protein, 31 aa, Equus caballus
EAEDPQVGQEELGGGPGLGGLQPLALAGPQQ

SEQ ID NO: 157 - protein, 31 aa, Equus caballus
EAEDPQVGEVELGGGPGLGGLQPLALAGPQQ

SEQ ID NO: 158 - protein, 31 aa, Equus caballus
EAEDPQVGQVELGGGPGLGGLQPLALAGPQQ

SEQ ID NO: 159 - protein, 31 aa, Chinchilla lanigera
ELEDPQVGQADPGVVPEAGRLQPLALEMTLQ

SEQ ID NO: 160 - protein, 31 aa, Cavia porcellus
ELEDPQVEQTELGMGLGAGGLQPLALEMALQ

SEQ ID NO: 161 - protein, 31 aa, Oryctolagus cuniculus
EVEELQVGQAELGGGPGAGGLQPSALELALQ

SEQ ID NO: 162 - protein, 31 aa, Canis lupus
EVEDLQVRDVELAGAPGEGGLQPLALEGALQ

SEQ ID NO: 163 - protein, 31 aa, Felis catus
EAEDLQGKDAELGEAPGAGGLQPSALEAPLQ

SEQ ID NO: 164 - protein, 26 aa, Bos taurus
EVEGPQVGALELAGGPGAGGLEGPPQ

SEQ ID NO: 165 - protein, 26 aa, Bos taurus
  Fleckvieh variant
EVEGPQVGALELAGGLGAGGLEGPPQ

SEQ ID NO: 166 - protein, 29 aa, Sus scrofa
EAENPQAGAVELGGGLGGLQALALEGPPQ

SEQ ID NO: 167 - protein, 29 aa, Mus musculus
EVEDPQVEQLELGGSPGDLQTLALEVARQ

SEQ ID NO: 168 - protein, 20 aa, Homo sapiens
PVLPVPPGFPPGPQIPVPRP

SEQ ID NO: 169 - protein, 11 aa, Homo sapiens
TCEEGFEPGPM

SEQ ID NO: 170 - protein, 41 aa, Homo sapiens
GLVPGVGVAPGVGVAPGVGVAPGVGLAPGVGVAPGVGVAPG

SEQ ID NO: 171 - protein, 20 aa, Homo sapiens
LPMGGIPGSAGSRPGGTGGN

SEQ ID NO: 172 - protein, 11 aa, Homo sapiens
NCNEGFEPGPM

SEQ ID NO: 173 - protein, 31 aa, Psammomys obesus
GVDDPQMPQLELGGSPGAGDLRALALEVARQ

SEQ ID NO: 174 - protein, 31 aa, Heterocephalus glaber
ELENLQVGQAEPGMGLEAGGLQPLAQELALQ

SEQ ID NO: 175 - protein, 18 aa, Homo sapiens
VGQVELGGGPGAGSLQPL

SEQ ID NO: 176 - protein, 14 aa, Homo sapiens
ELGGGPGAGSLQPL

SEQ ID NO: 177 - protein, 33 aa, Homo sapiens
CGNLSTCMLGTYTQDFNKFHTFPQTAIGVGAPG

SEQ ID NO: 178 - protein, 26 aa, Homo sapiens
MLGTYTQDFNKFHTFPQTAIGVGAPG

SEQ ID NO: 179 - protein, 18 aa, Homo sapiens
FNKFHTFPQTAIGVGAPG

SEQ ID NO: 180 - protein, 12 aa, Homo sapiens
FPQTAIGVGAPG

SEQ ID NO: 181 - protein, 8 aa, Homo sapiens
AIGVGAPG

SEQ ID NO: 182 - protein, 21 aa, Homo sapiens
SHPLGSPGSASDLETSGLQEQ

SEQ ID NO: 183 - protein, 19 aa, Homo sapiens
PLGSPGSASDLETSGLQEQ

SEQ ID NO: 184 - protein, 14 aa, Homo sapiens
PLGSPGSASDLETS

SEQ ID NO: 185 - protein, 9 aa, Homo sapiens
PLGSPGSAS

SEQ ID NO: 186 - protein, 6 aa, Homo sapiens
PLGSPG

SEQ ID NO: 187 - protein, 31 aa, Homo sapiens
EDVSAGEDCGPLPEGGPEPRSDGAKPGPREG

SEQ ID NO: 188 - protein, 26 aa, Homo sapiens
GEDCGPLPEGGPEPRSDGAKPGPREG

SEQ ID NO: 189 - protein, 21 aa, Homo sapiens
PLPEGGPEPRSDGAKPGPREG

SEQ ID NO: 190 - protein, 17 aa, Homo sapiens
PLPEGGPEPRSDGAKPG

SEQ ID NO: 191 - protein, 7 aa, Homo sapiens
SDGAKPG

SEQ ID NO: 192 - protein, 24 aa, Homo sapiens
RRNASSAGRLQGLAGGAPGQKECR

SEQ ID NO: 193 - protein, 16 aa, Homo sapiens
RLQGLAGGAPGQKECR

SEQ ID NO: 194 - protein, 20 aa, Homo sapiens
RRNASSAGRLQGLAGGAPGQ

SEQ ID NO: 195 - protein, 11 aa, Homo sapiens
LQGLAGGAPGQ

SEQ ID NO: 196 - protein, 6 aa, Homo sapiens
AGGAPG

SEQ ID NO: 197 - protein, 6 aa, Homo sapiens
YGYGPG

SEQ ID NO: 198 - protein, 6 aa, Homo sapiens
YGARPG

SEQ ID NO: 199 - protein, 6 aa, Homo sapiens
FGAVPG

SEQ ID NO: 200 - protein, 6 aa, Homo sapiens
GVGAPG

SEQ ID NO: 201 - protein, 6 aa, Homo sapiens
DGAKPG

SEQ ID NO: 202 - protein, 6 aa, Homo sapiens
QGMLPG

SEQ ID NO: 203 - protein, 10 aa, Homo sapiens
FGLVPGVGVA

SEQ ID NO: 204 - protein, 10 aa, Homo sapiens
GVAPGIGPGG

SEQ ID NO: 205 - protein, 28 aa, Homo sapiens
PPGAYPGQAPPGAYPGAPGAYPGAPAPG

SEQ ID NO: 206 - protein, 10 aa, Homo sapiens
TCEEGFEPGP

SEQ ID NO: 207 - protein, 10 aa, Homo sapiens
NPLGTIPGGN

SEQ ID NO: 208 - protein, 35 aa, Homo sapiens
RREAEDLQVGQVELGGGPGAGSLQPLALEGSLQKR

SEQ ID NO: 209 - protein, 18 aa, Homo sapiens
RVLQGVLPALPQVVCNYR

SEQ ID NO: 210 - protein, 38 aa, Homo sapiens
KRCGNLSTCMLGTYTQDFNKFHTFPQTAIGVGAPGKKR

SEQ ID NO: 211 - protein, 23 aa, Homo sapiens
RSHPLGSPGSASDLETSGLQEQR

SEQ ID NO: 212 - protein, 35 aa, Homo sapiens
KREDVSAGEDCGPLPEGGPEPRSDGAKPGPREGKR

SEQ ID NO: 213 - protein, 17 aa, Homo sapiens
RAAPLQGMLPGLLAPLR

SEQ ID NO: 214 - protein, 6 aa, Homo sapiens
FGLVPG

SEQ ID NO: 215 - protein, 6 aa, Homo sapiens
PGIGPG

SEQ ID NO: 216 - protein, 42 aa, Homo sapiens
VGVAPGVGVAPGVGVAPGVGLAPGVGVAPGVGVAPGVGVAPG

SEQ ID NO: 217 - protein, 16 aa, Homo sapiens
GVPGLGVGAGVPGLGV

SEQ ID NO: 218 - protein, 6 aa, Homo sapiens
GAGVPG

SEQ ID NO: 219 - protein, 5 aa, Homo sapiens
GISPE

SEQ ID NO: 220 - protein, 8 aa, Homo sapiens
LQGVLPAL

SEQ ID NO: 221 - protein, 5 aa, Homo sapiens
GVLPA

SEQ ID NO: 222 - protein, 10 aa, Homo sapiens
PGLGVGVGVP

SEQ ID NO: 223 - protein, 8 aa, Homo sapiens
GVGVGVPG

SEQ ID NO: 224 - protein, 6 aa, Homo sapiens
GVGVPG

SEQ ID NO: 225 - protein, 7 aa, Homo sapiens
GLVPGGP

SEQ ID NO: 226 - protein, 6 aa, Homo sapiens
PGFPPG

SEQ ID NO: 227 - protein, 6 aa, Homo sapiens
EKGPDP

SEQ ID NO: 228 - protein, 26 aa, Homo sapiens
EVEGPQVGALELAGGLGAGGLEGPPQ

SEQ ID NO: 229 - protein, 7 aa, Bos taurus
AGGLGAG

SEQ ID NO: 230 - protein, 7 aa, Bos taurus
AGGPGAG